European Patent Application EP 4 368 631 A1, published May 15, 2024. Title: A peptide with antiviral activity, Antiviral agents comprising the peptide and a method for producing the antiviral agent. Applicant: National University Corporation Tokyo Medical and Dental University. The sequence listing filed with the application follows.

SEQUENCE LISTING (66 sequences)

SEQ ID NO: 1 - protein, 20 aa, synthetic construct
  REGION 1..20: note = Synthetic peptide
DKEWILQKIYEIMRRLDEEG

SEQ ID NO: 2 - protein, 19 aa, synthetic construct
  REGION 1..19: note = Synthetic peptide
HGEASLRVSDLIYEFMKRD

SEQ ID NO: 3 - protein, 19 aa, synthetic construct
  REGION 1..19: note = Synthetic peptide
HGEASLRVSDLIYEFMKKD

SEQ ID NO: 4 - protein, 20 aa, synthetic construct
  REGION 1..20: note = Synthetic peptide
DKEWILQKIYEIMRLLDELG

SEQ ID NO: 5 - protein, 19 aa, synthetic construct
  REGION 1..19: note = Synthetic peptide
HAEASMRVSDLIYEFMKKD

SEQ ID NO: 6 - protein, 20 aa, synthetic construct
  REGION 1..20: note = Synthetic peptide
DKEWILQKIYEIMRKLDEDG

SEQ ID NO: 7 - protein, 20 aa, synthetic construct
  REGION 1..20: note = Synthetic peptide
DKEWALQKIYEIMRKLDEDG

SEQ ID NO: 8 - protein, 20 aa, synthetic construct
  REGION 1..20: note = Synthetic peptide
DKEWILQKIYEVMRKLDEDG

SEQ ID NO: 9 - protein, 19 aa, synthetic construct
  REGION 1..19: note = Synthetic peptide
HAEASMRASDLIYEFMKKD

SEQ ID NO: 10 - protein, 56 aa, synthetic construct
  REGION 1..56: note = Synthetic peptide
DKEWILQKIYEIMRLLDELGHAEASMRVSDLIYEFMKKGDERLLEEAERLLEEVER

SEQ ID NO: 11 - protein, 39 aa, synthetic construct
  REGION 1..39: note = Synthetic peptide
DKEWILQKIYEIMRLLDELGHAEASMRVSDLIYEFMKKG

SEQ ID NO: 12 - protein, 19 aa, synthetic construct
  REGION 1..19: note = Synthetic peptide
HAEASMRVSDLIYEFMKKG

SEQ ID NO: 13 - protein, 20 aa, synthetic construct
  REGION 1..20: note = Synthetic peptide
DKEWILQKIYENMRLLDELG

SEQ ID NO: 14 - protein, 19 aa, synthetic construct
  REGION 1..19: note = Synthetic peptide
HAEASMRVSDNIYEFMKKG

SEQ ID NO: 15 - protein, 20 aa, synthetic construct
  REGION 1..20: note = Synthetic peptide
DKEWILQKIYENMRKLDEDG

SEQ ID NO: 16 - protein, 20 aa, synthetic construct
  REGION 1..20: note = Synthetic peptide
DKEWILQKIYEAMRKLDEDG

SEQ ID NO: 17 - protein, 19 aa, synthetic construct
  REGION 1..19: note = Synthetic peptide
HAEASMRVSDAIYEFMKKG

SEQ ID NO: 18 - protein, 19 aa, synthetic construct
  REGION 1..19: note = Synthetic peptide
HAEASMRKSDDIYEFMKKG

SEQ ID NO: 19 - protein, 20 aa, synthetic construct
  REGION 1..20: note = Synthetic peptide
DKEWILQKIYENMRNLDELG

SEQ ID NO: 20 - protein, 20 aa, synthetic construct
  REGION 1..20: note = Synthetic peptide
DKEWILQKIYETMRKLDEDG

SEQ ID NO: 21 - protein, 20 aa, synthetic construct
  REGION 1..20: note = Synthetic peptide
DKEWILQKIYETMRNLDELG

SEQ ID NO: 22 - protein, 20 aa, synthetic construct
  REGION 1..20: note = Synthetic peptide
DREWILQKIYEIMRLLDELG

SEQ ID NO: 23 - protein, 19 aa, synthetic construct
  REGION 1..19: note = Synthetic peptide
HAESSMRVSDLIYEFMKKD

SEQ ID NO: 24 - protein, 19 aa, synthetic construct
  REGION 1..19: note = Synthetic peptide
HAEASMRVSDLIYEYMKKD

SEQ ID NO: 25 - protein, 20 aa, synthetic construct
  REGION 1..20: note = Synthetic peptide
DKEWILQKIYEEMRKLDEDG

SEQ ID NO: 26 - protein, 19 aa, synthetic construct
  REGION 1..19: note = Synthetic peptide
HAEASMRKSDLIYEFMKKD

SEQ ID NO: 27 - protein, 20 aa, synthetic construct
  REGION 1..20: note = Synthetic peptide
DKEWILQKIYEIMRRLDELG

SEQ ID NO: 28 - protein, 20 aa, synthetic construct
  REGION 1..20: note = Synthetic peptide
DKEWILQRIYEIMRLLDELG

SEQ ID NO: 29 - protein, 20 aa, synthetic construct
  REGION 1..20: note = Synthetic peptide
DKEWALQKIYEVMRKLDEDG

SEQ ID NO: 30 - protein, 19 aa, synthetic construct
  REGION 1..19: note = Synthetic peptide
HAEASMRVSELIYEFMKKD

SEQ ID NO: 31 - protein, 19 aa, synthetic construct
  REGION 1..19: note = Synthetic peptide
HAEASMRVSELIKEFMKKD

SEQ ID NO: 32 - protein, 19 aa, synthetic construct
  REGION 1..19: note = Synthetic peptide
HGEASMRVSDLIYEFMKKD

SEQ ID NO: 33 - protein, 19 aa, synthetic construct
  REGION 1..19: note = Synthetic peptide
HAQASMRVSDLIYEFMKKD

SEQ ID NO: 34 - protein, 19 aa, synthetic construct
  REGION 1..19: note = Synthetic peptide
HALASMRVSDLIYEFMKKD

SEQ ID NO: 35 - protein, 19 aa, synthetic construct
  REGION 1..19: note = Synthetic peptide
HAEASLRVSDLIYEFMKKD

SEQ ID NO: 36 - protein, 19 aa, synthetic construct
  REGION 1..19: note = Synthetic peptide
HAEASIRVSDLIYEFMKKD

SEQ ID NO: 37 - protein, 19 aa, synthetic construct
  REGION 1..19: note = Synthetic peptide
HAEASMRVADLIYEFMKKD

SEQ ID NO: 38 - protein, 19 aa, synthetic construct
  REGION 1..19: note = Synthetic peptide
HAEASMRVVDLIYEFMKKD

SEQ ID NO: 39 - protein, 19 aa, synthetic construct
  REGION 1..19: note = Synthetic peptide
HAEASMRVLDLIYEFMKKD

SEQ ID NO: 40 - protein, 19 aa, synthetic construct
  REGION 1..19: note = Synthetic peptide
HAEASMRVNDLIYEFMKKD

SEQ ID NO: 41 - protein, 19 aa, synthetic construct
  REGION 1..19: note = Synthetic peptide
HAEASMRVSALIYEFMKKD

SEQ ID NO: 42 - protein, 19 aa, synthetic construct
  REGION 1..19: note = Synthetic peptide
HAEASMRVSLLIYEFMKKD

SEQ ID NO: 43 - protein, 19 aa, synthetic construct
  REGION 1..19: note = Synthetic peptide
HAEASMRVSMLIYEFMKKD

SEQ ID NO: 44 - protein, 19 aa, synthetic construct
  REGION 1..19: note = Synthetic peptide
HAEASMRVSNLIYEFMKKD

SEQ ID NO: 45 - protein, 19 aa, synthetic construct
  REGION 1..19: note = Synthetic peptide
HAEASMRVSQLIYEFMKKD

SEQ ID NO: 46 - protein, 19 aa, synthetic construct
  REGION 1..19: note = Synthetic peptide
HAEASMRVSKLIYEFMKKD

SEQ ID NO: 47 - protein, 20 aa, synthetic construct
  REGION 1..20: note = Synthetic peptide
DKEWILQKIYEIKRRLDEEG

SEQ ID NO: 48 - protein, 20 aa, synthetic construct
  REGION 1..20: note = Synthetic peptide
DKEWILQKIYEIWRRLDEEG

SEQ ID NO: 49 - protein, 19 aa, synthetic construct
  REGION 1..19: note = Synthetic peptide
HGEASMRVSDLIYEFKKKD

SEQ ID NO: 50 - protein, 19 aa, synthetic construct
  REGION 1..19: note = Synthetic peptide
HGEASMRVSDLIYEFWKKD

SEQ ID NO: 51 - protein, 19 aa, synthetic construct
  REGION 1..19: note = Synthetic peptide
HGQASMRVSDLIYEFMKKD

SEQ ID NO: 52 - protein, 39 aa, synthetic construct
  REGION 1..39: note = Synthetic peptide
DKEWILQKIYEIMRKLDEDGHAEASMRVSDLIYEFMKKD

SEQ ID NO: 53 - protein, 39 aa, synthetic construct
  REGION 1..39: note = Synthetic peptide
DKEWILQKIYEIMRRLDEEGHAEASMRVSDLIYEFMKKD

SEQ ID NO: 54 - protein, 39 aa, synthetic construct
  REGION 1..39: note = Synthetic peptide
DKEWILQKIYEIMRRLDEEGHGEASLRVSDLIYEFMKKD

SEQ ID NO: 55 - protein, 39 aa, synthetic construct
  REGION 1..39: note = Synthetic peptide
DKEWILQKIYEIMRRLDEEGHGEASLRVSDLIYEFMKRD

SEQ ID NO: 56 - protein, 20 aa, synthetic construct
  REGION 1..20: note = Synthetic peptide
DKEWILQKIYEIMQRLDEEG

SEQ ID NO: 57 - protein, 19 aa, synthetic construct
  REGION 1..19: note = Synthetic peptide
HGEASLMVSDLIYEFMKRD

SEQ ID NO: 58 - protein, 39 aa, synthetic construct
  REGION 1..39: note = Synthetic peptide
DKEWILQKIYEIMQRLDEEGHGEASLMVSDLIYEFMKRD

SEQ ID NO: 59 - protein, 20 aa, synthetic construct
  REGION 1..20: note = Synthetic peptide
DKLWILQKIYEIMVRLDEEG

SEQ ID NO: 60 - protein, 39 aa, synthetic construct
  REGION 1..39: note = Synthetic peptide
DKLWILQKIYEIMVRLDEEGHGEASLMVSDLIYEFMKRD

SEQ ID NO: 61 - protein, 20 aa, synthetic construct
  REGION 1..20: note = Synthetic peptide
DKEWILYKIYEIMVRLDEEG

SEQ ID NO: 62 - protein, 39 aa, synthetic construct
  REGION 1..39: note = Synthetic peptide
DKEWILYKIYEIMVRLDEEGHGEASLMVSDLIYEFMKRD

SEQ ID NO: 63 - protein, 20 aa, synthetic construct
  REGION 1..20: note = Synthetic peptide
DKLWILQKIYEIMQRLDEEG

SEQ ID NO: 64 - protein, 39 aa, synthetic construct
  REGION 1..39: note = Synthetic peptide
DKLWILQKIYEIMQRLDEEGHGEASLMVSDLIYEFMKRD

SEQ ID NO: 65 - protein, 20 aa, synthetic construct
  REGION 1..20: note = Synthetic peptide
DKEWILYKIYEIMQRLDEEG

SEQ ID NO: 66 - protein, 39 aa, synthetic construct
  REGION 1..39: note = Synthetic peptide
DKEWILYKIYEIMQRLDEEGHGEASLMVSDLIYEFMKRD